European Patent Application EP 4 534 561 A1, published April 9, 2025. Title: BISPECIFIC CHIMERIC ANTIGEN RECEPTOR TARGETING BCMA-CD19 AND APPLICATION THEREOF. Applicant: Juventas Unicare Pharmaceutical (Beijing) Co., Ltd. The sequence listing filed with the application follows.

SEQUENCE LISTING (40 sequences)

SEQ ID NO: 1 - protein, 8 aa, synthetic construct
  REGION 1..8: note = BCMA VH CDR1
GFSLSTYH

SEQ ID NO: 2 - protein, 7 aa, synthetic construct
  REGION 1..7: note = BCMA VH CDR2
ISSSGST

SEQ ID NO: 3 - protein, 10 aa, synthetic construct
  REGION 1..10: note = BCMA VH CDR3
ARDLDYVIDL

SEQ ID NO: 4 - protein, 7 aa, synthetic construct
  REGION 1..7: note = BCMA VL CDR1
PSVYNNY

SEQ ID NO: 5 - skipped

SEQ ID NO: 6 - protein, 11 aa, synthetic construct
  REGION 1..11: note = BCMA VL CDR3
AGTYVSGDRRA

SEQ ID NO: 7 - protein, 8 aa, synthetic construct
  REGION 1..8: note = CD19 VH CDR1
GYAFSSYW

SEQ ID NO: 8 - protein, 8 aa, synthetic construct
  REGION 1..8: note = CD19 VH CDR2
IYPGDGDT

SEQ ID NO: 9 - protein, 15 aa, synthetic construct
  REGION 1..15: note = CD19 VH CDR3
ARKTISSVVDFYFDY

SEQ ID NO: 10 - protein, 6 aa, synthetic construct
  REGION 1..6: note = CD19 VL CDR1
QNVGTN

SEQ ID NO: 11 - skipped

SEQ ID NO: 12 - protein, 9 aa, synthetic construct
  REGION 1..9: note = CD19 VL CDR3
QQYNRYPYT

SEQ ID NO: 13 - protein, 116 aa, synthetic construct
  REGION 1..116: note = BCMA VH
EVQLVESGGGLVQPGGSLRLSCTASGFSLSTYHMTWVRQAPGKGLEWIGVISSSGSTYYASWAKGRFTISRDNSKNTVYLQMNSLRAEDTAVYFCARDLDYVIDLWGPGTLVTVSS

SEQ ID NO: 14 - protein, 110 aa, synthetic construct
  REGION 1..110: note = BCMA VL
EIVMTQSPSTLSASVGDRVIINCQSSPSVYNNYLSWYQQKPGKAPKLLIYETSTLASGVPSRFSGSGSGAEFTLTISSLQPDDFATYYCAGTYVSGDRRAFGQGTKLTVL

SEQ ID NO: 15 - protein, 114 aa, synthetic construct
  REGION 1..114: note = BCMA VH
QSVEESGGRLVTPGTPLTLTCTASGFSLSTYHMTWVRQAPGKGLEWIGVISSSGSTYYASWAKGRFTISKTSSTTVDLKMTSLTTEDTATYFCARDLDYVIDLWGQGTLVTVSS

SEQ ID NO: 16 - protein, 110 aa, synthetic construct
  REGION 1..110: note = BCMA VL
AQVLTQTPSSVSSAVGGTVTINCQSSPSVYNNYLSWFQQKPGQPPKLLIYETSTLPSGVPSRFSASGSGTQFTLTISGVQCDDAATYYCAGTYVSGDRRAFGGGTEVVVK

SEQ ID NO: 17 - protein, 122 aa, synthetic construct
  REGION 1..122: note = CD19 VH
QVQLQQSGAELVRPGSSVKISCKASGYAFSSYWMNWVKQRPGQGLEWIGQIYPGDGDTNYNGKFKGQATLTADKSSSTAYMQLSGLTSEDSAVYFCARKTISSVVDFYFDYWGQGTTLTVSS

SEQ ID NO: 18 - protein, 108 aa, synthetic construct
  REGION 1..108: note = CD19 VL
DIVLTQSPKFMSTSVGDRVSVTCKASQNVGTNVAWYQQKPGQSPKPLIYSATYRNSGVPDRFTGSGSGTDFTLTITNVQSKDLADYFCQQYNRYPYTSGGGTKLEIKR

SEQ ID NO: 19 - protein, 481 aa, synthetic construct
  REGION 1..481: note = Loop CD19-BCMAscFv
EIVMTQSPSTLSASVGDRVIINCQSSPSVYNNYLSWYQQKPGKAPKLLIYETSTLASGVPSRFSGSGSGAEFTLTISSLQPDDFATYYCAGTYVSGDRRAFGQGTKLTVLGGGGSDIVLTQSPKFMSTSVGDRVSVTCKASQNVGTNVAWYQQKPGQSPKPLIYSATYRNSGVPDRFTGSGSGTDFTLTITNVQSKDLADYFCQQYNRYPYTSGGGTKLEIKRGGGGSGGGGSGGGGSQVQLQQSGAELVRPGSSVKISCKASGYAFSSYWMNWVKQRPGQGLEWIGQIYPGDGDTNYNGKFKGQATLTADKSSSTAYMQLSGLTSEDSAVYFCARKTISSVVDFYFDYWGQGTTLTVSSGGGGSEVQLVESGGGLVQPGGSLRLSCTASGFSLSTYHMTWVRQAPGKGLEWIGVISSSGSTYYASWAKGRFTISRDNSKNTVYLQMNSLRAEDTAVYFCARDLDYVIDLWGPGTLVTVSS

SEQ ID NO: 20 - protein, 481 aa, synthetic construct
  REGION 1..481: note = Loop BCMA-CD19scFv
DIVLTQSPKFMSTSVGDRVSVTCKASQNVGTNVAWYQQKPGQSPKPLIYSATYRNSGVPDRFTGSGSGTDFTLTITNVQSKDLADYFCQQYNRYPYTSGGGTKLEIKRGGGGSEIVMTQSPSTLSASVGDRVIINCQSSPSVYNNYLSWYQQKPGKAPKLLIYETSTLASGVPSRFSGSGSGAEFTLTISSLQPDDFATYYCAGTYVSGDRRAFGQGTKLTVLGGGGSGGGGSGGGGSEVQLVESGGGLVQPGGSLRLSCTASGFSLSTYHMTWVRQAPGKGLEWIGVISSSGSTYYASWAKGRFTISRDNSKNTVYLQMNSLRAEDTAVYFCARDLDYVIDLWGPGTLVTVSSGGGGSQVQLQQSGAELVRPGSSVKISCKASGYAFSSYWMNWVKQRPGQGLEWIGQIYPGDGDTNYNGKFKGQATLTADKSSSTAYMQLSGLTSEDSAVYFCARKTISSVVDFYFDYWGQGTTLTVSS

SEQ ID NO: 21 - protein, 45 aa, synthetic construct
TTTPAPRPPTPAPTIASQPLSLRPEACRPAAGGAVHTRGLDFACD

SEQ ID NO: 22 - protein, 24 aa, synthetic construct
IYIWAPLAGTCGVLLLSLVITLYC

SEQ ID NO: 23 - protein, 112 aa, synthetic construct
RVKFSRSADAPAYQQGQNQLYNELNLGRREEYDVLDKRRGRDPEMGGKPRRKNPQEGLYNELQKDKMAEAYSEIGMKGERRRGKGHDGLYQGLSTATKDTYDALHMQALPPR

SEQ ID NO: 24 - protein, 42 aa, synthetic construct
KRGRKKLLYIFKQPFMRPVQTTQEEDGCSCRFPEEEEGGCEL

SEQ ID NO: 25 - protein, 21 aa, synthetic construct
MALPVTALLLPLALLLHAARP

SEQ ID NO: 26 - protein, 745 aa, synthetic construct
  REGION 1..745: note = Tan CD19-BCMA
MALPVTALLLPLALLLHAARPDIVLTQSPKFMSTSVGDRVSVTCKASQNVGTNVAWYQQKPGQSPKPLIYSATYRNSGVPDRFTGSGSGTDFTLTITNVQSKDLADYFCQQYNRYPYTSGGGTKLEIKRGGGGSGGGGSGGGGSQVQLQQSGAELVRPGSSVKISCKASGYAFSSYWMNWVKQRPGQGLEWIGQIYPGDGDTNYNGKFKGQATLTADKSSSTAYMQLSGLTSEDSAVYFCARKTISSVVDFYFDYWGQGTTLTVSSEAAAKEAAAKEAAAKEIVMTQSPSTLSASVGDRVIINCQSSPSVYNNYLSWYQQKPGKAPKLLIYETSTLASGVPSRFSGSGSGAEFTLTISSLQPDDFATYYCAGTYVSGDRRAFGQGTKLTVLGGGGSGGGGSGGGGSEVQLVESGGGLVQPGGSLRLSCTASGFSLSTYHMTWVRQAPGKGLEWIGVISSSGSTYYASWAKGRFTISRDNSKNTVYLQMNSLRAEDTAVYFCARDLDYVIDLWGPGTLVTVSSTTTPAPRPPTPAPTIASQPLSLRPEACRPAAGGAVHTRGLDFACDIYIWAPLAGTCGVLLLSLVITLYCKRGRKKLLYIFKQPFMRPVQTTQEEDGCSCRFPEEEEGGCELRVKFSRSADAPAYQQGQNQLYNELNLGRREEYDVLDKRRGRDPEMGGKPRRKNPQEGLYNELQKDKMAEAYSEIGMKGERRRGKGHDGLYQGLSTATKDTYDALHMQALPPR

SEQ ID NO: 27 - protein, 745 aa, synthetic construct
  REGION 1..745: note = Tan BCMA-CD19
MALPVTALLLPLALLLHAARPEIVMTQSPSTLSASVGDRVIINCQSSPSVYNNYLSWYQQKPGKAPKLLIYETSTLASGVPSRFSGSGSGAEFTLTISSLQPDDFATYYCAGTYVSGDRRAFGQGTKLTVLGGGGSGGGGSGGGGSEVQLVESGGGLVQPGGSLRLSCTASGFSLSTYHMTWVRQAPGKGLEWIGVISSSGSTYYASWAKGRFTISRDNSKNTVYLQMNSLRAEDTAVYFCARDLDYVIDLWGPGTLVTVSSEAAAKEAAAKEAAAKDIVLTQSPKFMSTSVGDRVSVTCKASQNVGTNVAWYQQKPGQSPKPLIYSATYRNSGVPDRFTGSGSGTDFTLTITNVQSKDLADYFCQQYNRYPYTSGGGTKLEIKRGGGGSGGGGSGGGGSQVQLQQSGAELVRPGSSVKISCKASGYAFSSYWMNWVKQRPGQGLEWIGQIYPGDGDTNYNGKFKGQATLTADKSSSTAYMQLSGLTSEDSAVYFCARKTISSVVDFYFDYWGQGTTLTVSSTTTPAPRPPTPAPTIASQPLSLRPEACRPAAGGAVHTRGLDFACDIYIWAPLAGTCGVLLLSLVITLYCKRGRKKLLYIFKQPFMRPVQTTQEEDGCSCRFPEEEEGGCELRVKFSRSADAPAYQQGQNQLYNELNLGRREEYDVLDKRRGRDPEMGGKPRRKNPQEGLYNELQKDKMAEAYSEIGMKGERRRGKGHDGLYQGLSTATKDTYDALHMQALPPR

SEQ ID NO: 28 - protein, 725 aa, synthetic construct
  REGION 1..725: note = Loop CD19-BCMA
MALPVTALLLPLALLLHAARPEIVMTQSPSTLSASVGDRVIINCQSSPSVYNNYLSWYQQKPGKAPKLLIYETSTLASGVPSRFSGSGSGAEFTLTISSLQPDDFATYYCAGTYVSGDRRAFGQGTKLTVLGGGGSDIVLTQSPKFMSTSVGDRVSVTCKASQNVGTNVAWYQQKPGQSPKPLIYSATYRNSGVPDRFTGSGSGTDFTLTITNVQSKDLADYFCQQYNRYPYTSGGGTKLEIKRGGGGSGGGGSGGGGSQVQLQQSGAELVRPGSSVKISCKASGYAFSSYWMNWVKQRPGQGLEWIGQIYPGDGDTNYNGKFKGQATLTADKSSSTAYMQLSGLTSEDSAVYFCARKTISSVVDFYFDYWGQGTTLTVSSGGGGSEVQLVESGGGLVQPGGSLRLSCTASGFSLSTYHMTWVRQAPGKGLEWIGVISSSGSTYYASWAKGRFTISRDNSKNTVYLQMNSLRAEDTAVYFCARDLDYVIDLWGPGTLVTVSSTTTPAPRPPTPAPTIASQPLSLRPEACRPAAGGAVHTRGLDFACDIYIWAPLAGTCGVLLLSLVITLYCKRGRKKLLYIFKQPFMRPVQTTQEEDGCSCRFPEEEEGGCELRVKFSRSADAPAYQQGQNQLYNELNLGRREEYDVLDKRRGRDPEMGGKPRRKNPQEGLYNELQKDKMAEAYSEIGMKGERRRGKGHDGLYQGLSTATKDTYDALHMQALPPR

SEQ ID NO: 29 - protein, 725 aa, synthetic construct
  REGION 1..725: note = Loop BCMA-CD19
MALPVTALLLPLALLLHAARPDIVLTQSPKFMSTSVGDRVSVTCKASQNVGTNVAWYQQKPGQSPKPLIYSATYRNSGVPDRFTGSGSGTDFTLTITNVQSKDLADYFCQQYNRYPYTSGGGTKLEIKRGGGGSEIVMTQSPSTLSASVGDRVIINCQSSPSVYNNYLSWYQQKPGKAPKLLIYETSTLASGVPSRFSGSGSGAEFTLTISSLQPDDFATYYCAGTYVSGDRRAFGQGTKLTVLGGGGSGGGGSGGGGSEVQLVESGGGLVQPGGSLRLSCTASGFSLSTYHMTWVRQAPGKGLEWIGVISSSGSTYYASWAKGRFTISRDNSKNTVYLQMNSLRAEDTAVYFCARDLDYVIDLWGPGTLVTVSSGGGGSQVQLQQSGAELVRPGSSVKISCKASGYAFSSYWMNWVKQRPGQGLEWIGQIYPGDGDTNYNGKFKGQATLTADKSSSTAYMQLSGLTSEDSAVYFCARKTISSVVDFYFDYWGQGTTLTVSSTTTPAPRPPTPAPTIASQPLSLRPEACRPAAGGAVHTRGLDFACDIYIWAPLAGTCGVLLLSLVITLYCKRGRKKLLYIFKQPFMRPVQTTQEEDGCSCRFPEEEEGGCELRVKFSRSADAPAYQQGQNQLYNELNLGRREEYDVLDKRRGRDPEMGGKPRRKNPQEGLYNELQKDKMAEAYSEIGMKGERRRGKGHDGLYQGLSTATKDTYDALHMQALPPR

SEQ ID NO: 30 - protein, 992 aa, synthetic construct
  REGION 1..992: note = CD19-2A-BCMA
MALPVTALLLPLALLLHAARPDIVLTQSPKFMSTSVGDRVSVTCKASQNVGTNVAWYQQKPGQSPKPLIYSATYRNSGVPDRFTGSGSGTDFTLTITNVQSKDLADYFCQQYNRYPYTSGGGTKLEIKRGGGGSGGGGSGGGGSQVQLQQSGAELVRPGSSVKISCKASGYAFSSYWMNWVKQRPGQGLEWIGQIYPGDGDTNYNGKFKGQATLTADKSSSTAYMQLSGLTSEDSAVYFCARKTISSVVDFYFDYWGQGTTLTVSSTTTPAPRPPTPAPTIASQPLSLRPEACRPAAGGAVHTRGLDFACDIYIWAPLAGTCGVLLLSLVITLYCKRGRKKLLYIFKQPFMRPVQTTQEEDGCSCRFPEEEEGGCELRVKFSRSADAPAYQQGQNQLYNELNLGRREEYDVLDKRRGRDPEMGGKPRRKNPQEGLYNELQKDKMAEAYSEIGMKGERRRGKGHDGLYQGLSTATKDTYDALHMQALPPREGRGSLLTCGDVEENPGPMALPVTALLLPLALLLHAARPEIVMTQSPSTLSASVGDRVIINCQSSPSVYNNYLSWYQQKPGKAPKLLIYETSTLASGVPSRFSGSGSGAEFTLTISSLQPDDFATYYCAGTYVSGDRRAFGQGTKLTVLGGGGSGGGGSGGGGSEVQLVESGGGLVQPGGSLRLSCTASGFSLSTYHMTWVRQAPGKGLEWIGVISSSGSTYYASWAKGRFTISRDNSKNTVYLQMNSLRAEDTAVYFCARDLDYVIDLWGPGTLVTVSSTTTPAPRPPTPAPTIASQPLSLRPEACRPAAGGAVHTRGLDFACDIYIWAPLAGTCGVLLLSLVITLYCKRGRKKLLYIFKQPFMRPVQTTQEEDGCSCRFPEEEEGGCELRVKFSRSADAPAYQQGQNQLYNELNLGRREEYDVLDKRRGRDPEMGGKPRRKNPQEGLYNELQKDKMAEAYSEIGMKGERRRGKGHDGLYQGLSTATKDTYDALHMQALPPR

SEQ ID NO: 31 - protein, 992 aa, synthetic construct
  REGION 1..992: note = BCMA-2A-CD19
MALPVTALLLPLALLLHAARPEIVMTQSPSTLSASVGDRVIINCQSSPSVYNNYLSWYQQKPGKAPKLLIYETSTLASGVPSRFSGSGSGAEFTLTISSLQPDDFATYYCAGTYVSGDRRAFGQGTKLTVLGGGGSGGGGSGGGGSEVQLVESGGGLVQPGGSLRLSCTASGFSLSTYHMTWVRQAPGKGLEWIGVISSSGSTYYASWAKGRFTISRDNSKNTVYLQMNSLRAEDTAVYFCARDLDYVIDLWGPGTLVTVSSTTTPAPRPPTPAPTIASQPLSLRPEACRPAAGGAVHTRGLDFACDIYIWAPLAGTCGVLLLSLVITLYCKRGRKKLLYIFKQPFMRPVQTTQEEDGCSCRFPEEEEGGCELRVKFSRSADAPAYQQGQNQLYNELNLGRREEYDVLDKRRGRDPEMGGKPRRKNPQEGLYNELQKDKMAEAYSEIGMKGERRRGKGHDGLYQGLSTATKDTYDALHMQALPPREGRGSLLTCGDVEENPGPMALPVTALLLPLALLLHAARPDIVLTQSPKFMSTSVGDRVSVTCKASQNVGTNVAWYQQKPGQSPKPLIYSATYRNSGVPDRFTGSGSGTDFTLTITNVQSKDLADYFCQQYNRYPYTSGGGTKLEIKRGGGGSGGGGSGGGGSQVQLQQSGAELVRPGSSVKISCKASGYAFSSYWMNWVKQRPGQGLEWIGQIYPGDGDTNYNGKFKGQATLTADKSSSTAYMQLSGLTSEDSAVYFCARKTISSVVDFYFDYWGQGTTLTVSSTTTPAPRPPTPAPTIASQPLSLRPEACRPAAGGAVHTRGLDFACDIYIWAPLAGTCGVLLLSLVITLYCKRGRKKLLYIFKQPFMRPVQTTQEEDGCSCRFPEEEEGGCELRVKFSRSADAPAYQQGQNQLYNELNLGRREEYDVLDKRRGRDPEMGGKPRRKNPQEGLYNELQKDKMAEAYSEIGMKGERRRGKGHDGLYQGLSTATKDTYDALHMQALPPR

SEQ ID NO: 32 - protein, 489 aa, synthetic construct
  REGION 1..489: note = CD19 CAR
MALPVTALLLPLALLLHAARPDIVLTQSPKFMSTSVGDRVSVTCKASQNVGTNVAWYQQKPGQSPKPLIYSATYRNSGVPDRFTGSGSGTDFTLTITNVQSKDLADYFCQQYNRYPYTSGGGTKLEIKRGGGGSGGGGSGGGGSQVQLQQSGAELVRPGSSVKISCKASGYAFSSYWMNWVKQRPGQGLEWIGQIYPGDGDTNYNGKFKGQATLTADKSSSTAYMQLSGLTSEDSAVYFCARKTISSVVDFYFDYWGQGTTLTVSSTTTPAPRPPTPAPTIASQPLSLRPEACRPAAGGAVHTRGLDFACDIYIWAPLAGTCGVLLLSLVITLYCKRGRKKLLYIFKQPFMRPVQTTQEEDGCSCRFPEEEEGGCELRVKFSRSADAPAYQQGQNQLYNELNLGRREEYDVLDKRRGRDPEMGGKPRRKNPQEGLYNELQKDKMAEAYSEIGMKGERRRGKGHDGLYQGLSTATKDTYDALHMQALPPR

SEQ ID NO: 33 - protein, 485 aa, synthetic construct
  REGION 1..485: note = BCMA CAR
MALPVTALLLPLALLLHAARPEIVMTQSPSTLSASVGDRVIINCQSSPSVYNNYLSWYQQKPGKAPKLLIYETSTLASGVPSRFSGSGSGAEFTLTISSLQPDDFATYYCAGTYVSGDRRAFGQGTKLTVLGGGGSGGGGSGGGGSEVQLVESGGGLVQPGGSLRLSCTASGFSLSTYHMTWVRQAPGKGLEWIGVISSSGSTYYASWAKGRFTISRDNSKNTVYLQMNSLRAEDTAVYFCARDLDYVIDLWGPGTLVTVSSTTTPAPRPPTPAPTIASQPLSLRPEACRPAAGGAVHTRGLDFACDIYIWAPLAGTCGVLLLSLVITLYCKRGRKKLLYIFKQPFMRPVQTTQEEDGCSCRFPEEEEGGCELRVKFSRSADAPAYQQGQNQLYNELNLGRREEYDVLDKRRGRDPEMGGKPRRKNPQEGLYNELQKDKMAEAYSEIGMKGERRRGKGHDGLYQGLSTATKDTYDALHMQALPPR

SEQ ID NO: 34 - protein, 15 aa, synthetic construct
GGGGSGGGGSGGGGS

SEQ ID NO: 35 - protein, 5 aa, synthetic construct
GGGGS

SEQ ID NO: 36 - protein, 15 aa, synthetic construct
EAAAKEAAAKEAAAK

SEQ ID NO: 37 - DNA, 348 bp, synthetic construct
  misc_feature 1..348: note = SEQ ID NO:13BCMA VH
  source 1..348: mol_type = other DNA
gaagtgcagctggtggagtccggcggtggactggtgcaaccgggaggctcactcagattgtcatgcaccgcctctggctttagtctctccacctatcatatgacttgggtgaggcaggcacccggcaagggcctggaatggatcggcgtgatctcttccagcggtagcacctattacgcctcttgggcgaagggcaggtttaccatcagccgcgacaacagcaagaataccgtttacctgcagatgaatagcctgagggccgaagacacggcggtctatttctgtgcacgggaccttgactacgttattgacctgtggggccctgggaccctcgtaactgtgagcagc

SEQ ID NO: 38 - DNA, 330 bp, synthetic construct
  misc_feature 1..330: note = SEQ ID NO:14BCMA VL
  source 1..330: mol_type = other DNA
gagatcgtgatgacccagtccccaagtacactgagcgcctccgtgggcgaccgcgtgatcataaactgtcaaagctcaccctctgtttacaacaattacctgtcttggtatcaacagaagcccggtaaggcccccaaactgctcatttacgagacatccaccctggcatccggggtgccaagccgcttctccgggagtgggtctggcgccgagttcaccctgaccatatcttccctgcagcccgacgacttcgcaacgtactattgcgccggaacctatgtaagtggggatagacgcgccttcgggcagggcacgaagttgaccgtgctg

SEQ ID NO: 39 - DNA, 366 bp, synthetic construct
  misc_feature 1..366: note = SEQ ID NO:17CD19 VH
  source 1..366: mol_type = other DNA
caagtgcaactgcaacagagcggagccgaactggtgagacccggaagcagcgtgaagatcagctgcaaggcttccggctacgcctttagcagctactggatgaactgggtgaagcagagacctggacagggactggaatggatcggccagatttaccctggagacggcgacacaaactacaacggcaagttcaagggccaagctacactgaccgccgacaaaagcagcagcaccgcctatatgcagctgagcggactgaccagcgaagatagcgctgtgtacttctgcgccagaaagaccatcagcagcgtggtggacttctacttcgactactggggacaaggcaccaccctgacagtgagcagc

SEQ ID NO: 40 - DNA, 324 bp, synthetic construct
  misc_feature 1..324: note = SEQ ID NO:18CD19 VL
  source 1..324: mol_type = other DNA
gatattgtgctgacccagagccccaagttcatgagcaccagcgtgggcgatagagtgagcgtgacctgcaaggcaagccagaacgtgggaacaaacgtggcctggtaccaacagaaacccggccaaagccctaagcccctgatttacagcgccacctacagaaatagcggcgtgcccgacagatttacaggaagcggcagcggaaccgatttcacactgaccatcaccaacgtgcagagcaaagacctggccgactacttctgccagcagtacaacagatacccctacaccagcggaggaggaacaaagctggagatcaagaga